European Patent Application EP 4 559 932 A1, published May 28, 2025. Title: 多特异性抗体及其用途. Applicant: 明慧医药（杭州）有限公司. The sequence listing filed with the application follows.

SEQUENCE LISTING (35 sequences)

SEQ ID NO: 1 - protein, 118 aa, synthetic construct
  source 1..118: note; note (original language) = PD-1单域抗体VHH
QVQLVESGGGLVQPGGSLRLSCATSGSRRSIYAMGWFRQAPGKGLEFVAGIGWAYATTYYADSVKGRFTISRDNTKNTLYLQMNSLRAEDTAVYYCAADLDHSGFDYWGQGTLVTVSS

SEQ ID NO: 2 - protein, 5 aa, synthetic construct
  source 1..5: note; note (original language) = PD-1单域抗体 CDR1
IYAMG

SEQ ID NO: 3 - protein, 17 aa, synthetic construct
  source 1..17: note; note (original language) = PD-1单域抗体 CDR2
GIGWAYATTYYADSVKG

SEQ ID NO: 4 - protein, 9 aa, synthetic construct
  source 1..9: note; note (original language) = PD-1单域抗体 CDR3
DLDHSGFDY

SEQ ID NO: 5 - protein, 123 aa, synthetic construct
  source 1..123: note = Bevacizumab (mutant) VH
EVQLVQSGGGVVQPGGSLRLSCAASGYTFTNYGMNWVRQAPGKGLEWVGWINTYTGEPTYAADFKRRFTFSLDTSKSTAYLQMNSLRAEDTAVYYCAKYPHYYGSSHWYFDVWGQGTLVTVSS

SEQ ID NO: 6 - protein, 107 aa, synthetic construct [sequence omitted]

SEQ ID NO: 7 - protein, 5 aa, synthetic construct
  source 1..5: note = Bevacizumab (mutant) CDR-H1
NYGMN

SEQ ID NO: 8 - protein, 17 aa, synthetic construct
  source 1..17: note = Bevacizumab (mutant) CDR-H2
WINTYTGEPTYAADFKR

SEQ ID NO: 9 - protein, 14 aa, synthetic construct
  source 1..14: note = Bevacizumab (mutant) CDR-H3
YPHYYGSSHWYFDV

SEQ ID NO: 10 - protein, 11 aa, synthetic construct
  source 1..11: note = Bevacizumab (mutant) CDR-L1
SASQDISNYLN

SEQ ID NO: 11 - protein, 7 aa, synthetic construct
  source 1..7: note = Bevacizumab (mutant) CDR-L2
FTSSLHS

SEQ ID NO: 12 - protein, 9 aa, synthetic construct
  source 1..9: note = Bevacizumab (mutant) CDR-L3
QQYSTVPWT

SEQ ID NO: 13 - protein, 123 aa, synthetic construct [sequence omitted]

SEQ ID NO: 14 - protein, 107 aa, synthetic construct [sequence omitted]

SEQ ID NO: 15 - protein, 5 aa, synthetic construct
  source 1..5: note = Ranibizumab CDR-H1
HYGMN

SEQ ID NO: 16 - protein, 17 aa, synthetic construct
  source 1..17: note = Ranibizumab CDR-H2
WINTYTGEPTYAADFKR

SEQ ID NO: 17 - protein, 14 aa, synthetic construct
  source 1..14: note = Ranibizumab CDR-H3
YPYYYGTSHWYFDV

SEQ ID NO: 18 - protein, 11 aa, synthetic construct
  source 1..11: note = Ranibizumab CDR-L1
SASQDISNYLN

SEQ ID NO: 19 - protein, 7 aa, synthetic construct
  source 1..7: note = Ranibizumab CDR-L2
FTSSLHS

SEQ ID NO: 20 - protein, 9 aa, synthetic construct
  source 1..9: note = Ranibizumab CDR-L3
QQYSTVPWT

SEQ ID NO: 21 - protein, 330 aa, synthetic construct
  source 1..330: note; note (original language) = 重链恒定区
ASTKGPSVFPLAPSSKSTSGGTAALGCLVKDYFPEPVTVSWNSGALTSGVHTFPAVLQSSGLYSLSSVVTVPSSSLGTQTYICNVNHKPSNTKVDKKVEPKSCDKTHTCPPCPAPEAAGGPSVFLFPPKPKDTLMISRTPEVTCVVVDVSHEDPEVKFNWYVDGVEVHNAKTKPREEQYNSTYRVVSVLTVLHQDWLNGKEYKCKVSNKALPAPIEKTISKAKGQPREPQVYTLPPSREEMTKNQVSLTCLVKGFYPSDIAVEWESNGQPENNYKTTPPVLDSDGSFFLYSKLTVDKSRWQQGNVFSCSVMHEALHNHYTQKSLSLSPGK

SEQ ID NO: 22 - protein, 107 aa, synthetic construct [sequence omitted]

SEQ ID NO: 23 - protein, 586 aa, synthetic construct
  source 1..586: note = 162-17-HC
QVQLVESGGGLVQPGGSLRLSCATSGSRRSIYAMGWFRQAPGKGLEFVAGIGWAYATTYYADSVKGRFTISRDNTKNTLYLQMNSLRAEDTAVYYCAADLDHSGFDYWGQGTLVTVSSGGGGSGGGGSGGGGSEVQLVQSGGGVVQPGGSLRLSCAASGYTFTNYGMNWVRQAPGKGLEWVGWINTYTGEPTYAADFKRRFTFSLDTSKSTAYLQMNSLRAEDTAVYYCAKYPHYYGSSHWYFDVWGQGTLVTVSSASTKGPSVFPLAPSSKSTSGGTAALGCLVKDYFPEPVTVSWNSGALTSGVHTFPAVLQSSGLYSLSSVVTVPSSSLGTQTYICNVNHKPSNTKVDKKVEPKSCDKTHTCPPCPAPEAAGGPSVFLFPPKPKDTLMISRTPEVTCVVVDVSHEDPEVKFNWYVDGVEVHNAKTKPREEQYNSTYRVVSVLTVLHQDWLNGKEYKCKVSNKALPAPIEKTISKAKGQPREPQVYTLPPSREEMTKNQVSLTCLVKGFYPSDIAVEWESNGQPENNYKTTPPVLDSDGSFFLYSKLTVDKSRWQQGNVFSCSVMHEALHNHYTQKSLSLSPGK

SEQ ID NO: 24 - protein, 214 aa, synthetic construct
  source 1..214: note = 162-17-LC
DIQMTQSPSSLSASVGDRVTITCSASQDISNYLNWYQQKPGKAPKVLIYFTSSLHSGVPSRFSGSGSGTDFTLTISSLQPEDFATYYCQQYSTVPWTFGQGTKVEIKRTVAAPSVFIFPPSDEQLKSGTASVVCLLNNFYPREAKVQWKVDNALQSGNSQESVTEQDSKDSTYSLSSTLTLSKADYEKHKVYACEVTHQGLSSPVTKSFNRGEC

SEQ ID NO: 25 - protein, 453 aa, synthetic construct
  source 1..453: note = 162-18-HC
EVQLVQSGGGVVQPGGSLRLSCAASGYTFTNYGMNWVRQAPGKGLEWVGWINTYTGEPTYAADFKRRFTFSLDTSKSTAYLQMNSLRAEDTAVYYCAKYPHYYGSSHWYFDVWGQGTLVTVSSASTKGPSVFPLAPSSKSTSGGTAALGCLVKDYFPEPVTVSWNSGALTSGVHTFPAVLQSSGLYSLSSVVTVPSSSLGTQTYICNVNHKPSNTKVDKKVEPKSCDKTHTCPPCPAPEAAGGPSVFLFPPKPKDTLMISRTPEVTCVVVDVSHEDPEVKFNWYVDGVEVHNAKTKPREEQYNSTYRVVSVLTVLHQDWLNGKEYKCKVSNKALPAPIEKTISKAKGQPREPQVYTLPPSREEMTKNQVSLTCLVKGFYPSDIAVEWESNGQPENNYKTTPPVLDSDGSFFLYSKLTVDKSRWQQGNVFSCSVMHEALHNHYTQKSLSLSPGK

SEQ ID NO: 26 - protein, 347 aa, synthetic construct
  source 1..347: note = 162-18-LC
QVQLVESGGGLVQPGGSLRLSCATSGSRRSIYAMGWFRQAPGKGLEFVAGIGWAYATTYYADSVKGRFTISRDNTKNTLYLQMNSLRAEDTAVYYCAADLDHSGFDYWGQGTLVTVSSGGGGSGGGGSGGGGSDIQMTQSPSSLSASVGDRVTITCSASQDISNYLNWYQQKPGKAPKVLIYFTSSLHSGVPSRFSGSGSGTDFTLTISSLQPEDFATYYCQQYSTVPWTFGQGTKVEIKRTVAAPSVFIFPPSDEQLKSGTASVVCLLNNFYPREAKVQWKVDNALQSGNSQESVTEQDSKDSTYSLSSTLTLSKADYEKHKVYACEVTHQGLSSPVTKSFNRGEC

SEQ ID NO: 27 - protein, 586 aa, synthetic construct
  source 1..586: note = 162-19-HC
EVQLVQSGGGVVQPGGSLRLSCAASGYTFTNYGMNWVRQAPGKGLEWVGWINTYTGEPTYAADFKRRFTFSLDTSKSTAYLQMNSLRAEDTAVYYCAKYPHYYGSSHWYFDVWGQGTLVTVSSASTKGPSVFPLAPSSKSTSGGTAALGCLVKDYFPEPVTVSWNSGALTSGVHTFPAVLQSSGLYSLSSVVTVPSSSLGTQTYICNVNHKPSNTKVDKKVEPKSCDKTHTCPPCPAPEAAGGPSVFLFPPKPKDTLMISRTPEVTCVVVDVSHEDPEVKFNWYVDGVEVHNAKTKPREEQYNSTYRVVSVLTVLHQDWLNGKEYKCKVSNKALPAPIEKTISKAKGQPREPQVYTLPPSREEMTKNQVSLTCLVKGFYPSDIAVEWESNGQPENNYKTTPPVLDSDGSFFLYSKLTVDKSRWQQGNVFSCSVMHEALHNHYTQKSLSLSPGKGGGGSGGGGSGGGGSQVQLVESGGGLVQPGGSLRLSCATSGSRRSIYAMGWFRQAPGKGLEFVAGIGWAYATTYYADSVKGRFTISRDNTKNTLYLQMNSLRAEDTAVYYCAADLDHSGFDYWGQGTLVTVSS

SEQ ID NO: 28 - protein, 214 aa, synthetic construct; identical to SEQ ID NO: 24
  source 1..214: note = 162-19-LC

SEQ ID NO: 29 - protein, 586 aa, synthetic construct
  source 1..586: note = 162-20-HC
QVQLVESGGGLVQPGGSLRLSCATSGSRRSIYAMGWFRQAPGKGLEFVAGIGWAYATTYYADSVKGRFTISRDNTKNTLYLQMNSLRAEDTAVYYCAADLDHSGFDYWGQGTLVTVSSGGGGSGGGGSGGGGSEVQLVESGGGLVQPGGSLRLSCAASGYDFTHYGMNWVRQAPGKGLEWVGWINTYTGEPTYAADFKRRFTFSLDTSKSTAYLQMNSLRAEDTAVYYCAKYPYYYGTSHWYFDVWGQGTLVTVSSASTKGPSVFPLAPSSKSTSGGTAALGCLVKDYFPEPVTVSWNSGALTSGVHTFPAVLQSSGLYSLSSVVTVPSSSLGTQTYICNVNHKPSNTKVDKKVEPKSCDKTHTCPPCPAPEAAGGPSVFLFPPKPKDTLMISRTPEVTCVVVDVSHEDPEVKFNWYVDGVEVHNAKTKPREEQYNSTYRVVSVLTVLHQDWLNGKEYKCKVSNKALPAPIEKTISKAKGQPREPQVYTLPPSREEMTKNQVSLTCLVKGFYPSDIAVEWESNGQPENNYKTTPPVLDSDGSFFLYSKLTVDKSRWQQGNVFSCSVMHEALHNHYTQKSLSLSPGK

SEQ ID NO: 30 - protein, 214 aa, synthetic construct
  source 1..214: note = 162-20-LC
DIQLTQSPSSLSASVGDRVTITCSASQDISNYLNWYQQKPGKAPKVLIYFTSSLHSGVPSRFSGSGSGTDFTLTISSLQPEDFATYYCQQYSTVPWTFGQGTKVEIKRTVAAPSVFIFPPSDEQLKSGTASVVCLLNNFYPREAKVQWKVDNALQSGNSQESVTEQDSKDSTYSLSSTLTLSKADYEKHKVYACEVTHQGLSSPVTKSFNRGEC

SEQ ID NO: 31 - protein, 453 aa, synthetic construct
  source 1..453: note = 162-21-HC
EVQLVESGGGLVQPGGSLRLSCAASGYDFTHYGMNWVRQAPGKGLEWVGWINTYTGEPTYAADFKRRFTFSLDTSKSTAYLQMNSLRAEDTAVYYCAKYPYYYGTSHWYFDVWGQGTLVTVSSASTKGPSVFPLAPSSKSTSGGTAALGCLVKDYFPEPVTVSWNSGALTSGVHTFPAVLQSSGLYSLSSVVTVPSSSLGTQTYICNVNHKPSNTKVDKKVEPKSCDKTHTCPPCPAPEAAGGPSVFLFPPKPKDTLMISRTPEVTCVVVDVSHEDPEVKFNWYVDGVEVHNAKTKPREEQYNSTYRVVSVLTVLHQDWLNGKEYKCKVSNKALPAPIEKTISKAKGQPREPQVYTLPPSREEMTKNQVSLTCLVKGFYPSDIAVEWESNGQPENNYKTTPPVLDSDGSFFLYSKLTVDKSRWQQGNVFSCSVMHEALHNHYTQKSLSLSPGK

SEQ ID NO: 32 - protein, 347 aa, synthetic construct
  source 1..347: note = 162-21-LC
QVQLVESGGGLVQPGGSLRLSCATSGSRRSIYAMGWFRQAPGKGLEFVAGIGWAYATTYYADSVKGRFTISRDNTKNTLYLQMNSLRAEDTAVYYCAADLDHSGFDYWGQGTLVTVSSGGGGSGGGGSGGGGSDIQLTQSPSSLSASVGDRVTITCSASQDISNYLNWYQQKPGKAPKVLIYFTSSLHSGVPSRFSGSGSGTDFTLTISSLQPEDFATYYCQQYSTVPWTFGQGTKVEIKRTVAAPSVFIFPPSDEQLKSGTASVVCLLNNFYPREAKVQWKVDNALQSGNSQESVTEQDSKDSTYSLSSTLTLSKADYEKHKVYACEVTHQGLSSPVTKSFNRGEC

SEQ ID NO: 33 - protein, 586 aa, synthetic construct
  source 1..586: note = 162-22-HC
EVQLVESGGGLVQPGGSLRLSCAASGYDFTHYGMNWVRQAPGKGLEWVGWINTYTGEPTYAADFKRRFTFSLDTSKSTAYLQMNSLRAEDTAVYYCAKYPYYYGTSHWYFDVWGQGTLVTVSSASTKGPSVFPLAPSSKSTSGGTAALGCLVKDYFPEPVTVSWNSGALTSGVHTFPAVLQSSGLYSLSSVVTVPSSSLGTQTYICNVNHKPSNTKVDKKVEPKSCDKTHTCPPCPAPEAAGGPSVFLFPPKPKDTLMISRTPEVTCVVVDVSHEDPEVKFNWYVDGVEVHNAKTKPREEQYNSTYRVVSVLTVLHQDWLNGKEYKCKVSNKALPAPIEKTISKAKGQPREPQVYTLPPSREEMTKNQVSLTCLVKGFYPSDIAVEWESNGQPENNYKTTPPVLDSDGSFFLYSKLTVDKSRWQQGNVFSCSVMHEALHNHYTQKSLSLSPGKGGGGSGGGGSGGGGSQVQLVESGGGLVQPGGSLRLSCATSGSRRSIYAMGWFRQAPGKGLEFVAGIGWAYATTYYADSVKGRFTISRDNTKNTLYLQMNSLRAEDTAVYYCAADLDHSGFDYWGQGTLVTVSS

SEQ ID NO: 34 - protein, 214 aa, synthetic construct; identical to SEQ ID NO: 30
  source 1..214: note = 162-22-LC

SEQ ID NO: 35 - protein, 15 aa, synthetic construct
  source 1..15: note = Linker
GGGGSGGGGSGGGGS